European Patent Application EP 4 112 637 A1, published January 4, 2023. Title: Polypeptide compounds and use thereof in the prevention or treatment of diabetes or diabetic complications. Applicant: Shenzhen Turier Biotech. Co.,Ltd. The sequence listing filed with the application follows.

SEQUENCE LISTING (28 sequences)

SEQ ID NO: 1 - protein, 39 aa, Artificial
  MISC_FEATURE (2)..(2): X=Aib
  MISC_FEATURE (10)..(10): A side chain of Lys is linked to -PEG2-PEG2-γGlu-CO(CH2)18CO2H
  MISC_FEATURE (16)..(16): X=Aib
HXQGTFTSDKSKYLEXKAAQDFVEWLKAGGPSSGAPPPS

SEQ ID NO: 2 - protein, 39 aa, Artificial; identical to SEQ ID NO: 1
  MISC_FEATURE (2)..(2): X=D-Ser
  MISC_FEATURE (10)..(10): A side chain of Lys is linked to PEG2-PEG2-CO(CH2)18CO2H
  MISC_FEATURE (16)..(16): X=Aib

SEQ ID NO: 3 - protein, 39 aa, Artificial; identical to SEQ ID NO: 1
  MISC_FEATURE (2)..(2): X=D-Ser
  MISC_FEATURE (10)..(10): A side chain of Lys is linked to -PEG2-PEG2-γGlu-CO(CH2)18CO2H
  MISC_FEATURE (16)..(16): X=Aib

SEQ ID NO: 4 - protein, 39 aa, Artificial; identical to SEQ ID NO: 1
  MISC_FEATURE (2)..(2): X=D-Ser
  MISC_FEATURE (10)..(10): A side chain of Lys is linked to -PEG2-PEG2-γGlu-CO(CH2)16CO2H
  MISC_FEATURE (16)..(16): X=Aib

SEQ ID NO: 5 - protein, 39 aa, Artificial; identical to SEQ ID NO: 1
  MISC_FEATURE (2)..(2): X=D-Ser
  MISC_FEATURE (10)..(10): A side chain of Lys is linked to -PEG2-PEG2-γGlu-CO(CH2)18CH3
  MISC_FEATURE (16)..(16): X=Aib

SEQ ID NO: 6 - protein, 39 aa, Artificial
  MISC_FEATURE (2)..(2): X=D-Ser
  MISC_FEATURE (10)..(10): A side chain of Lys is linked to -PEG2-PEG2-γGlu-CO(CH2)18CO2H
  MISC_FEATURE (23)..(23): X=Iva
  MISC_FEATURE (35)..(35): X=Aib
HXQGTFTSDKSKYLDERAAQDFXQWLLDGGPSSGXPPPS

SEQ ID NO: 7 - protein, 39 aa, Artificial
  MISC_FEATURE (2)..(2): X=D-Ser
  MISC_FEATURE (10)..(10): A side chain of Lys is linked to -PEG2-PEG2-γGlu-CO(CH2)18CO2H
  MISC_FEATURE (23)..(23): X=Iva
HXQGTFTSDKSKYLDERAAQDFXQWLLEGGPSSGAPPPS

SEQ ID NO: 8 - protein, 39 aa, Artificial; identical to SEQ ID NO: 6
  MISC_FEATURE (2)..(2): X=Aib
  MISC_FEATURE (10)..(10): A side chain of Lys is linked to -PEG2-PEG2-γGlu-CO(CH2)18CO2H
  MISC_FEATURE (23)..(23): X=Iva
  MISC_FEATURE (35)..(35): X=Aib

SEQ ID NO: 9 - protein, 39 aa, Artificial; identical to SEQ ID NO: 6
  MISC_FEATURE (2)..(2): X=Aib
  MISC_FEATURE (10)..(10): A side chain of Lys is linked to -PEG2-PEG2-γGlu-CO(CH2)16CO2H
  MISC_FEATURE (23)..(23): X=Iva
  MISC_FEATURE (35)..(35): X=Aib

SEQ ID NO: 10 - protein, 39 aa, Artificial; identical to SEQ ID NO: 6
  MISC_FEATURE (2)..(2): X=Aib
  MISC_FEATURE (10)..(10): A side chain of Lys is linked to -PEG2-PEG2-γGlu-CO(CH2)18CH3
  MISC_FEATURE (23)..(23): X=Iva
  MISC_FEATURE (35)..(35): X=Aib

SEQ ID NO: 11 - protein, 39 aa, Artificial; identical to SEQ ID NO: 6
  MISC_FEATURE (2)..(2): X=Aib
  MISC_FEATURE (10)..(10): A side chain of Lys is linked to -PEG2-PEG2-CO(CH2)18CH3
  MISC_FEATURE (23)..(23): X=Iva
  MISC_FEATURE (35)..(35): X=Aib

SEQ ID NO: 12 - protein, 39 aa, Artificial; identical to SEQ ID NO: 6
  MISC_FEATURE (2)..(2): X=D-Ser
  MISC_FEATURE (10)..(10): A side chain of Lys is linked to -PEG2-PEG2-γGlu-CO(CH2)18CO2H
  MISC_FEATURE (23)..(23): X=Iva
  MISC_FEATURE (35)..(35): X=Aib

SEQ ID NO: 13 - protein, 39 aa, Artificial; identical to SEQ ID NO: 1
  MISC_FEATURE (2)..(2): X=D-Ser
  MISC_FEATURE (10)..(10): A side chain of Lys is linked to -Gly-Gly-Ser-Gly-Ser-Gly-γGlu-CO(CH2)18-COOH
  MISC_FEATURE (16)..(16): X=Aib

SEQ ID NO: 14 - protein, 39 aa, Artificial; identical to SEQ ID NO: 1
  MISC_FEATURE (2)..(2): X=D-Ser
  MISC_FEATURE (10)..(10): A side chain of Lys is linked to -Gly-Gly-Ser-Gly-Ser-Gly-γGlu-CO(CH2)18-COOH
  MISC_FEATURE (16)..(16): X=Aib

SEQ ID NO: 15 - protein, 39 aa, Artificial; identical to SEQ ID NO: 6
  MISC_FEATURE (2)..(2): X=Aib
  MISC_FEATURE (10)..(10): A side chain of Lys is linked to -Gly-Gly-Ser-Gly-Ser-Gly-γGlu-CO(CH2)18-COOH
  MISC_FEATURE (23)..(23): X=Iva
  MISC_FEATURE (35)..(35): X=Aib

SEQ ID NO: 16 - protein, 39 aa, Artificial; identical to SEQ ID NO: 6
  MISC_FEATURE (2)..(2): X=Aib
  MISC_FEATURE (10)..(10): A side chain of Lys is linked to -Gly-Gly-Ser-Gly-Ser-Gly-γGlu-CO(CH2)18-COOH
  MISC_FEATURE (23)..(23): X=Iva
  MISC_FEATURE (35)..(35): X=Aib

SEQ ID NO: 17 - protein, 40 aa, Artificial
  MISC_FEATURE (2)..(2): X=D-Ser
  MISC_FEATURE (16)..(16): A side chain of Lys is linked to -PEG2-PEG2-γGlu-CO(CH2)14CH3
HXQGTFTSDYSKYLDKRRAQDFVQWLMNTGGPSSGAPPPS

SEQ ID NO: 18 - protein, 40 aa, Artificial
  MISC_FEATURE (2)..(2): X=D-Ser
  MISC_FEATURE (16)..(16): A side chain of Lys is linked to -PEG2-PEG2-γGlu-CO(CH2)14CH3
HXQGTFTSDYSKYLDKRRAQDFVQWLLNTGGPSSGAPPPS

SEQ ID NO: 19 - protein, 40 aa, Artificial
  MISC_FEATURE (2)..(2): X=D-Ser
  MISC_FEATURE (12)..(12): A side chain of Lys is linked to -PEG2-PEG2-CO(CH2)16CO2H
  MISC_FEATURE (16)..(16): X=Aib
HXQGTFTSDYSKKLDXRRAQDFVQWLMNTGGPSSGAPPPS

SEQ ID NO: 20 - protein, 40 aa, Artificial; identical to SEQ ID NO: 17
  MISC_FEATURE (2)..(2): X=D-Ser
  MISC_FEATURE (16)..(16): A side chain of Lys is linked to -(PEG2-PEG2-γGlu-CO(CH2)14CH3

SEQ ID NO: 21 - protein, 38 aa, Artificial
  MISC_FEATURE (2)..(2): Xaa=aminoisobutyric acid
HXQGTFTSDKSKYLDEQAAQDFVQWLLDGPSSGAPPPS

SEQ ID NO: 22 - protein, 39 aa, Artificial
HSQGTFTSDKSKYLDSQAAQDFVQWLMNGGPSSGAPPPS

SEQ ID NO: 23 - protein, 39 aa, Artificial
HSQGTFTSDKSKYLDEEAAQDFVQWLMNGGPSSGAPPPS

SEQ ID NO: 24 - protein, 39 aa, Artificial
HSQGTFTSDKSKYLDEQAAQDFVQWLMNGGPSSGAPPPS

SEQ ID NO: 25 - protein, 39 aa, Artificial
HSQGTFTSDKSKYLDERAAQDFVQWLMNTGPSSGAPPPS

SEQ ID NO: 26 - protein, 39 aa, Artificial
HSQGTFTSDKSKYLDSRAAQDFVQWLMNTGPSSGAPPPS

SEQ ID NO: 27 - protein, 30 aa, Artificial
  MISC_FEATURE (2)..(2): X=D-Ser
  MISC_FEATURE (13)..(13): A side chain of Lys is linked to -PEG2-PEG2-γGlu-CO(CH2)17COOH
HXQGTFTSDYSKKLDSERARDFVAWLVAGG

SEQ ID NO: 28 - protein, 39 aa, Artificial
  MISC_FEATURE (2)..(2): X=D-Ser
  MISC_FEATURE (14)..(14): A side chain of Lys is linked to -CO(CH2)14CH3
HXQGTFTSDLSKQKESKAAQDFIEWLKAGGPSSGAPPPS